European Patent Application EP 4 790 150 A1, published August 12, 2026. Title: INTEGRATIVE APPROACH FOR IDENTIFYING TUMOR-SPECIFIC ANTIGENS IN NSCLC USING RNA SEQUENCING AND MASS SPECTROMETRY-BASED IMMUNOPEPTIDOMICS AND RELATED METHODS. Applicant: VITO. Application EP. The sequence listing filed with the application follows.

SEQUENCE LISTING (102 sequences)

SEQ ID NO: 1 - protein, 9 aa, Homo sapiens
FEEGGGIAM

SEQ ID NO: 2 - protein, 9 aa, Homo sapiens
ITDEPPPGL

SEQ ID NO: 3 - protein, 13 aa, Homo sapiens
RKGGSYSQAASSD

SEQ ID NO: 4 - protein, 9 aa, Homo sapiens
ALAPAPVEV

SEQ ID NO: 5 - protein, 9 aa, Homo sapiens
EELKLRQQL

SEQ ID NO: 6 - protein, 9 aa, Homo sapiens
KTSDVVLKR

SEQ ID NO: 7 - protein, 9 aa, Homo sapiens
TLSPEIITV

SEQ ID NO: 8 - protein, 9 aa, Homo sapiens
VSYGGTVSL

SEQ ID NO: 9 - protein, 10 aa, Homo sapiens
RMAGIGIREA

SEQ ID NO: 10 - protein, 8 aa, Homo sapiens
LPQKGLKI

SEQ ID NO: 11 - protein, 9 aa, Homo sapiens
EHIDSLSSF

SEQ ID NO: 12 - protein, 11 aa, Homo sapiens
AIYHGSFSTKK

SEQ ID NO: 13 - protein, 19 aa, Homo sapiens
FHKYTRRDDKIDKPSLLTM

SEQ ID NO: 14 - protein, 22 aa, Homo sapiens
IDMFHKYTRRDDKIDKPSLLTM

SEQ ID NO: 15 - protein, 14 aa, Homo sapiens
FQKWASVVVPSGEE

SEQ ID NO: 16 - protein, 16 aa, Homo sapiens
SPDHIFLPIPNWEHKE

SEQ ID NO: 17 - protein, 18 aa, Homo sapiens
TEEGSISIYKSSQGAKKV

SEQ ID NO: 18 - protein, 10 aa, Homo sapiens
VNETLREAEK

SEQ ID NO: 19 - protein, 15 aa, Homo sapiens
NVQMSSTVIKSSHPE

SEQ ID NO: 20 - protein, 15 aa, Homo sapiens
PPLSFSQTNVQMSST

SEQ ID NO: 21 - protein, 16 aa, Homo sapiens
IEEFDFIISQLGYEPN

SEQ ID NO: 22 - protein, 9 aa, Homo sapiens
TVAEVIQSV

SEQ ID NO: 23 - protein, 9 aa, Homo sapiens
ILDEVIMGY

SEQ ID NO: 24 - protein, 9 aa, Homo sapiens
YSDKYGLGY

SEQ ID NO: 25 - protein, 10 aa, Homo sapiens
QELDGVFQKL

SEQ ID NO: 26 - protein, 8 aa, Homo sapiens
FPRLKSKL

SEQ ID NO: 27 - protein, 9 aa, Homo sapiens
KLKEVKEFL

SEQ ID NO: 28 - protein, 9 aa, Homo sapiens
RYFDEPVEL

SEQ ID NO: 29 - protein, 9 aa, Homo sapiens
VLLDGVQNL

SEQ ID NO: 30 - protein, 9 aa, Homo sapiens
RESPIFKQF

SEQ ID NO: 31 - protein, 10 aa, Homo sapiens
RSDETQRVFK

SEQ ID NO: 32 - protein, 8 aa, Homo sapiens
LPQKGLKI

SEQ ID NO: 33 - protein, 9 aa, Homo sapiens
EHIDSLSSF

SEQ ID NO: 34 - protein, 9 aa, Homo sapiens
ITDEPPPGL

SEQ ID NO: 35 - protein, 11 aa, Homo sapiens
HHAVEEEESRF

SEQ ID NO: 36 - protein, 10 aa, Homo sapiens
SVAPPTIPSA

SEQ ID NO: 37 - protein, 11 aa, Homo sapiens
IPRRPRALDGL

SEQ ID NO: 38 - protein, 10 aa, Homo sapiens
ETPGESASSL

SEQ ID NO: 39 - protein, 9 aa, Homo sapiens
AHDMAQVFL

SEQ ID NO: 40 - protein, 9 aa, Homo sapiens
NAKLRVDQL

SEQ ID NO: 41 - protein, 10 aa, Homo sapiens
PLGAGNTVLR

SEQ ID NO: 42 - protein, 13 aa, Homo sapiens
RKGGSYSQAASSD

SEQ ID NO: 43 - protein, 9 aa, Homo sapiens
HHSIPVEGF

SEQ ID NO: 44 - protein, 9 aa, Homo sapiens
RELEQRAAL

SEQ ID NO: 45 - protein, 9 aa, Homo sapiens
APTPVSPVL

SEQ ID NO: 46 - protein, 11 aa, Homo sapiens
EEAEYYFQKEF

SEQ ID NO: 47 - protein, 8 aa, Homo sapiens
AEDVGLYY

SEQ ID NO: 48 - protein, 11 aa, Homo sapiens
RVFGGGTKLTV

SEQ ID NO: 49 - protein, 9 aa, Homo sapiens
GQGPPTAGV

SEQ ID NO: 50 - protein, 9 aa, Homo sapiens
AEGITATVF

SEQ ID NO: 51 - protein, 9 aa, Homo sapiens
DSIPLSTGY

SEQ ID NO: 52 - protein, 10 aa, Homo sapiens
SFGGSYGGSF

SEQ ID NO: 53 - protein, 10 aa, Homo sapiens
RMAGIGIREA

SEQ ID NO: 54 - protein, 9 aa, Homo sapiens
RLKFAVEEI

SEQ ID NO: 55 - protein, 9 aa, Homo sapiens
VPHTNPPAY

SEQ ID NO: 56 - protein, 9 aa, Homo sapiens
AELGVSMQY

SEQ ID NO: 57 - protein, 9 aa, Homo sapiens
TVFQGMLRK

SEQ ID NO: 58 - protein, 8 aa, Homo sapiens
RQFIVRKV

SEQ ID NO: 59 - protein, 9 aa, Homo sapiens
AVMDAAVFL

SEQ ID NO: 60 - protein, 9 aa, Homo sapiens
ALAPAPVEV

SEQ ID NO: 61 - protein, 9 aa, Homo sapiens
KTSDVVLKR

SEQ ID NO: 62 - protein, 9 aa, Homo sapiens
METPAQLLL

SEQ ID NO: 63 - protein, 10 aa, Homo sapiens
TPTSGRTSVL

SEQ ID NO: 64 - protein, 8 aa, Homo sapiens
SVDDPLEY

SEQ ID NO: 65 - protein, 9 aa, Homo sapiens
IYIIGIFRN

SEQ ID NO: 66 - protein, 9 aa, Homo sapiens
APRPFGSVF

SEQ ID NO: 67 - protein, 9 aa, Homo sapiens
ILGEVINAL

SEQ ID NO: 68 - protein, 9 aa, Homo sapiens
RVTIVGDNL

SEQ ID NO: 69 - protein, 9 aa, Homo sapiens
FEEGENSLL

SEQ ID NO: 70 - protein, 9 aa, Homo sapiens
HTNEVVAIK

SEQ ID NO: 71 - protein, 9 aa, Homo sapiens
RPLRGLRAL

SEQ ID NO: 72 - protein, 12 aa, Homo sapiens
RPRPGSGLGRVM

SEQ ID NO: 73 - protein, 9 aa, Homo sapiens
AHDSNVLHI

SEQ ID NO: 74 - protein, 9 aa, Homo sapiens
TLSPEIITV

SEQ ID NO: 75 - protein, 9 aa, Homo sapiens
KFIEGNITY

SEQ ID NO: 76 - protein, 10 aa, Homo sapiens
WHDISDFLIY

SEQ ID NO: 77 - protein, 9 aa, Homo sapiens
RAAEQQRAY

SEQ ID NO: 78 - protein, 9 aa, Homo sapiens
GLLVGGAVS

SEQ ID NO: 79 - protein, 9 aa, Homo sapiens
NAAAAAAVY

SEQ ID NO: 80 - protein, 11 aa, Homo sapiens
SPRVPVSPLKF

SEQ ID NO: 81 - protein, 9 aa, Homo sapiens
LPSDDRGSL

SEQ ID NO: 82 - protein, 9 aa, Homo sapiens
LPQQPPLSL

SEQ ID NO: 83 - protein, 9 aa, Homo sapiens
THSLGNFSF

SEQ ID NO: 84 - protein, 9 aa, Homo sapiens
SPSETVNSL

SEQ ID NO: 85 - protein, 9 aa, Homo sapiens
LEFPDNDSL

SEQ ID NO: 86 - protein, 9 aa, Homo sapiens
APAKYSITF

SEQ ID NO: 87 - protein, 11 aa, Homo sapiens
AAAPAAAATAA

SEQ ID NO: 88 - protein, 9 aa, Homo sapiens
GPRGSLAVA

SEQ ID NO: 89 - protein, 9 aa, Homo sapiens
VSYGGTVSL

SEQ ID NO: 90 - protein, 14 aa, Homo sapiens
ITEEIYKTGLLSGL

SEQ ID NO: 91 - protein, 9 aa, Homo sapiens
RDVDPGEHY

SEQ ID NO: 92 - protein, 10 aa, Homo sapiens
RDVDPGEHYI

SEQ ID NO: 93 - protein, 12 aa, Homo sapiens
LKGKIGKVPVRF

SEQ ID NO: 94 - protein, 9 aa, Homo sapiens
LVDSGAQVS

SEQ ID NO: 95 - protein, 9 aa, Homo sapiens
PVGGSLEDE

SEQ ID NO: 96 - protein, 12 aa, Homo sapiens
DTFYIKTSTTVR

SEQ ID NO: 97 - protein, 9 aa, Homo sapiens
NVMLRKIAV

SEQ ID NO: 98 - protein, 9 aa, Homo sapiens
RTTEINFKV

SEQ ID NO: 99 - protein, 9 aa, Homo sapiens
AEYRLGPLL

SEQ ID NO: 100 - protein, 10 aa, Homo sapiens
APKPSSRPSL

SEQ ID NO: 101 - protein, 9 aa, Homo sapiens
PKPSSRPSL

SEQ ID NO: 102 - protein, 11 aa, Homo sapiens
RVYSPPEWISR